European Patent Application EP 4 144 756 A1, published March 8, 2023. Title: THERAPEUTIC TREATMENT OF SKIN DISEASE WITH RECOMBINANT COMMENSAL SKIN MICROORGANISMS. Applicant: AZITRA, INC. The sequence listing filed with the application follows.

SEQUENCE LISTING (35 sequences)

SEQ ID NO: 1 - protein, 4061 aa, Homo sapiens
MSTLLENIFAIINLFKQYSKKDKNTDTLSKKELKELLEKEFRQILKNPDDPDMVDVFMDHLDIDHNKKIDFTEFLLMVFKLAQAYYESTRKENLPISGHKHRKHSHHDKHEDNKQEENKENRKRPSSLERRNNRKGNKGRSKSPRETGGKRHESSSEKKERKGYSPTHREEEYGKNHHNSSKKEKNKTENTRLGDNRKRLSERLEEKEDNEEGVYDYENTGRMTQKWIQSGHIATYYTIQDEAYDTTDSLLEENKIYERSRSSDGKSSSQVNRSRHENTSQVPLQESRTRKRRGSRVSQDRDSEGHSEDSERHSGSASRNHHGSAWEQSRDGSRHPRSHDEDRASHGHSADSSRQSGTRHAETSSRGQTASSHEQARSSPGERHGSGHQQSADSSRHSATGRGQASSAVSDRGHRGSSGSQASDSEGHSENSDTQSVSGHGKAGLRQQSHQESTRGRSGERSGRSGSSLYQVSTHEQPDSAHGRTGTSTGGRQGSHHEQARDSSRHSASQEGQDTIRGHPGSSRGGRQGSHHEQSVNRSGHSGSHHSHTTSQGRSDASHGQSGSRSASRQTRNEEQSGDGTRHSGSRHHEASSQADSSRHSQVGQGQSSGPRTSRNQGSSVSQDSDSQGHSEDSERWSGSASRNHHGSAQEQSRDGSRHPRSHHEDRAGHGHSADSSRKSGTRHTQNSSSGQAASSHEQARSSAGERHGSRHQLQSADSSRHSGTGHGQASSAVRDSGHRGSSGSQATDSEGHSEDSDTQSVSGHGQAGHHQQSHQESARDRSGERSRRSGSFLYQVSTHKQSESSHGWTGPSTGVRQGSHHEQARDNSRHSASQDGQDTIRGHPGSSRRGRQGSHHEQSVDRSGHSGSHHSHTTSQGRSDASRGQSGSRSASRTTRNEEQSRDGSRHSGSRHHEASSHADISRHSQAGQGQSEGSRTSRRQGSSVSQDSDSEGHSEDSERWSGSASRNHRGSAQEQSRHGSRHPRSHHEDRAGHGHSADSSRQSGTPHAETSSGGQAASSHEQARSSPGERHGSRHQQSADSSRHSGIPRRQASSAVRDSGHWGSSGSQASDSEGHSEESDTQSVSGHGQDGPHQQSHQESARDWSGGRSGRSGSFIYQVSTHEQSESAHGRTRTSTGRRQGSHHEQARDSSRHSASQEGQDTIRAHPGSRRGGRQGSHHEQSVDRSGHSGSHHSHTTSQGRSDASHGQSGSRSASRQTRKDKQSGDGSRHSGSRHHEAASWADSSRHSQVGQEQSSGSRTSRHQGSSVSQDSDSERHSDDSERLSGSASRNHHGSSREQSRDGSRHPGFHQEDRASHGHSADSSRQSGTHHTESSSHGQAVSSHEQARSSPGERHGSRHQQSADSSRHSGIGHRQASSAVRDSGHRGSSGSQVTNSEGHSEDSDTQSVSAHGQAGPHQQSHKESARGQSGESSGRSRSFLYQVSSHEQSESTHGQTAPSTGGRQGSRHEQARNSSRHSASQDGQDTIRGHPGSSRGGRQGSYHEQSVDRSGHSGYHHSHTTPQGRSDASHGQSGPRSASRQTRNEEQSGDGSRHSGSRHHEPSTRAGSSRHSQVGQGESAGSKTSRRQGSSVSQDRDSEGHSEDSERRSESASRNHYGSAREQSRHGSRNPRSHQEDRASHGHSAESSRQSGTRHAETSSGGQAASSQEQARSSPGERHGSRHQQSADSSTDSGTGRRQDSSVVGDSGNRGSSGSQASDSEGHSEESDTQSVSAHGQAGPHQQSHQESTRGQSGERSGRSGSFLYQVSTHEQSESAHGRTGPSTGGRQRSRHEQARDSSRHSASQEGQDTIRGHPGSSRGGRQGSHYEQSVDSSGHSGSHHSHTTSQERSDVSRGQSGSRSVSRQTRNEKQSGDGSRHSGSRHHEASSRADSSRHSQVGQGQSSGPRTSRNQGSSVSQDSDSQGHSEDSERWSGSASRNHLGSAWEQSRDGSRHPGSHHEDRAGHGHSADSSRQSGTRHTESSSRGQAASSHEQARSSAGERHGSHHQLQSADSSRHSGIGHGQASSAVRDSGHRGYSGSQASDSEGHSEDSDTQSVSAQGKAGPHQQSHKESARGQSGESSGRSGSFLYQVSTHEQSESTHGQSAPSTGGRQGSHYDQAQDSSRHSASQEGQDTIRGHPGPSRGGRQGSHQEQSVDRSGHSGSHHSHTTSQGRSDASRGQSGSRSASRKTYDKEQSGDGSRHSGSHHHEASSWADSSRHSLVGQGQSSGPRTSRPRGSSVSQDSDSEGHSEDSERRSGSASRNHHGSAQEQSRDGSRHPRSHHEDRAGHGHSAESSRQSGTHHAENSSGGQAASSHEQARSSAGERHGSHHQQSADSSRHSGIGHGQASSAVRDSGHRGSSGSQASDSEGHSEDSDTQSVSAHGQAGPHQQSHQESTRGRSAGRSGRSGSFLYQVSTHEQSESAHGRTGTSTGGRQGSHHKQARDSSRHSTSQEGQDTIHGHPGSSSGGRQGSHYEQLVDRSGHSGSHHSHTTSQGRSDASHGHSGSRSASRQTRNDEQSGDGSRHSGSRHHEASSRADSSGHSQVGQGQSEGPRTSRNWGSSFSQDSDSQGHSEDSERWSGSASRNHHGSAQEQLRDGSRHPRSHQEDRAGHGHSADSSRQSGTRHTQTSSGGQAASSHEQARSSAGERHGSHHQQSADSSRHSGIGHGQASSAVRDSGHRGYSGSQASDNEGHSEDSDTQSVSAHGQAGSHQQSHQESARGRSGETSGHSGSFLYQVSTHEQSESSHGWTGPSTRGRQGSRHEQAQDSSRHSASQDGQDTIRGHPGSSRGGRQGYHHEHSVDSSGHSGSHHSHTTSQGRSDASRGQSGSRSASRTTRNEEQSGDGSRHSGSRHHEASTHADISRHSQAVQGQSEGSRRSRRQGSSVSQDSDSEGHSEDSERWSGSASRNHHGSAQEQLRDGSRHPRSHQEDRAGHGHSADSSRQSGTRHTQTSSGGQAASSHEQARSSAGERHGSHHQQSADSSRHSGIGHGQASSAVRDSGHRGYSGSQASDNEGHSEDSDTQSVSAHGQAGSHQQSHQESARGRSGETSGHSGSFLYQVSTHEQSESSHGWTGPSTRGRQGSRHEQAQDSSRHSASQYGQDTIRGHPGSSRGGRQGYHHEHSVDSSGHSGSHHSHTTSQGRSDASRGQSGSRSASRTTRNEEQSGDSSRHSVSRHHEASTHADISRHSQAVQGQSEGSRRSRRQGSSVSQDSDSEGHSEDSERWSGSASRNHRGSVQEQSRHGSRHPRSHHEDRAGHGHSADRSRQSGTRHAETSSGGQAASSHEQARSSPGERHGSRHQQSADSSRHSGIPRGQASSAVRDSRHWGSSGSQASDSEGHSEESDTQSVSGHGQAGPHQQSHQESARDRSGGRSGRSGSFLYQVSTHEQSESAHGRTRTSTGRRQGSHHEQARDSSRHSASQEGQDTIRGHPGSSRRGRQGSHYEQSVDRSGHSGSHHSHTTSQGRSDASRGQSGSRSASRQTRNDEQSGDGSRHSWSHHHEASTQADSSRHSQSGQGQSAGPRTSRNQGSSVSQDSDSQGHSEDSERWSGSASRNHRGSAQEQSRDGSRHPTSHHEDRAGHGHSAESSRQSGTHHAENSSGGQAASSHEQARSSAGERHGSHHQQSADSSRHSGIGHGQASSAVRDSGHRGSSGSQASDSEGHSEDSDTQSVSAHGQAGPHQQSHQESTRGRSAGRSGRSGSFLYQVSTHEQSESAHGRAGPSTGGRQGSRHEQARDSSRHSASQEGQDTIRGHPGSRRGGRQGSYHEQSVDRSGHSGSHHSHTTSQGRSDASHGQSGSRSASRETRNEEQSGDGSRHSGSRHHEASTQADSSRHSQSGQGESAGSRRSRRQGSSVSQDSDSEAYPEDSERRSESASRNHHGSSREQSRDGSRHPGSSHRDTASHVQSSPVQSDSSTAKEHGHFSSLSQDSAYHSGIQSRGSPHSSSSYHYQSEGTERQKGQSGLVWRHGSYGSADYDYGESGFRHSQHGSVSYNSNPVVFKERSDICKASAFGKDHPRYYATYINKDPGLCGHSSDISKQLGFSQSQRYYYYE

SEQ ID NO: 2 - protein, 4061 aa, Homo sapiens; identical to SEQ ID NO: 1

SEQ ID NO: 3 - protein, 4061 aa, Homo sapiens; identical to SEQ ID NO: 1

SEQ ID NO: 4 - protein, 4061 aa, Homo sapiens; identical to SEQ ID NO: 1

SEQ ID NO: 5 - protein, 4061 aa, Homo sapiens; identical to SEQ ID NO: 1

SEQ ID NO: 6 - protein, 554 aa, Mus musculus
MSALLESITSMIEIFQQYSTSDKEEETLSKEELKELLEGQLQAVLKNPDDQDIAEVFMQMLDVDHDDKLDFAEYLLLVLKLAKAYYEASKNESFQTHGSNGRSKTDYKGLEEEGEEGNEQNLRRRHGGTDGKRKSDRTRSPNGKRGKRQESRCRSEGKDKHRREPEKHRHQQDSKRKQRHGSGSTERKDNRNKKNRQSKERNYDEIYDNGKYNEDWEASYNNCYYKTQNTTLDQREGNRRPRADSQKEPQSFHGQADNSDSEGGRQQSHSKPSPVRADQRRSRAGQAGSSKVSARSGSGGRGQSPDGSGRSSNRRDRPRQPSPSQSSDSQVHSGVQVEGRRGQSSSANRRAGSSSGSGVQGASAGGLAADASRRTGALQGQASAQGRAGSQGQAQGRVGSSADRQGRRGVSESQASDSEGQSDFSEGQAVGAHRQSGAGQRHEQRSSRGQYGSGFYPVYYYYEQEHSEEESDSQHGHQHEQQRGHQHQHQHEHEQPESGHRQQQSSGRGHQGAHQEQGRDSARSRGSNQGHSSSRHQADSPRVSVRSGSGGRGQ

SEQ ID NO: 7 - protein, 336 aa, Mus musculus
PDGSGRSSNRRDRPRQLSPSQSSDSQVHSGVQVEGRRGHSSSANRRAGSSSGSGVQGASAGGLAADASRRSGARQGQASAQGRAGSQGQAQGRVSSSADRQGRRGVSESRASDSEGHSDFSEGQAVGAHRQSGAGQRHEQRSSRGQHGSGYYYEQEHSEEESDSQHQHGHQHEQQRGHQHQHQHQHEHEQPESGHRQQQSSGRGHQGAHQEQGRDSARPRGSNQGHSSSRHQADSPRVSARSGSGGRGQSPDASGRSSNRRDRPRQPSPSQSSDSQVHSGVQVEAQRGQSSSANRRAGSSSGSGVQGAAASGQGGYESIFTAKHLDFNQSHSYYYY

SEQ ID NO: 8 - protein, 250 aa, Mus musculus
GGLAADASRRSGALQGQASAQGRAGSQGQAQGRVGSSADRQGRRGVSESQASDSEGHSDFSEGQAVGAHRQSGAGQRHEQRSSRGQHGSGYYYEQEHSEEESDSQHQHGHQHEQQRGHQHQHQHQHEHEQPESGHRQQQSSGRGHQGAHQEQGRDSARSRGSNQGHSSSRHQADSPRVSARSGSGGRGQSPDASGRSSNRRDRPRQPSPSQSSDSQVHSGVQVEGRRGQSSSANRRAGSSSSSGVQGASA

SEQ ID NO: 9 - protein, 255 aa, Mus musculus
GGLAADASRRSGARQGQASAQGRAGSQGQAQGRVGSSADRQGRRGVSESQASDSEGHSDFSEGQAVGAHRQSGAGQRHEQRSSRGQHGSGFYPVYYYYEQEHSEEESDSQHQHGHQHEQQRGHQHQHQHQHEHEQPESGHRQQQSSGRGHQGAHQEQGRDSARSRGSNQGHSSSRHQADSPRVSARSGSGGRGQSPDASGRSSNRRDRPRQPSPSQSSDSQVHSGVQVEGRRGQSSSANRRAGSSSGSGVQGASA

SEQ ID NO: 10 - protein, 4838 aa, Mus musculus
MSALLESITSMIEIFQQYSTSDKEEETLSKEELKELLEGQLQAVLKIIQLLDDYPKCFIVGADNVGSKQMQQIRMSLRGKAVVLMGKKTMMRKAIRGHLENNPALEKLLPHIRGNVGFVFTKEDLTEIRAMLLANKVPAAARVGAIAPCEVTMPAQNTGLGPEKISFFQALGITTRISRGTIEILSDVQLIKTGDKVGVSEATLLNMLNISPSSFGLIIQQVFDNGSIYNPEVLDITEQALHSRFLEGVHNVASVCLQIGYLTVDSVLHSFINGYKRVLALSVETEYTFPLAEKVKAFLANPSAFATAAITAAPAAATAPAKPENPDDQDIAEVFMQMLDVDHDDKLDFAEYLLLVLKLAKAYYEASKNESFQTHGSNGRSKTDYKGLEEEGEEGNKQNLRRRHGGTDGKRKSDRTRSPNGKRGKRQESRCRSEGKDKHRREPEKHRHQQDSKRKQRHGSGSTERKDNRNKKNRQSKERNYDEIYDNGKYNEDWEASYNNCYYKTQNTTLDQREGNRRPRADSQKEPQSSHGQADNSDSEGGRQQSHSKPSPVRADQRRSRAGQAGSSKVSARSGSGGRGQSPDGSGRSSNRRDRPRQPSPSQSSDSQVHSGVQVEGRRGQSSSANRRAGSSSGSGVQGASAGGLAADASRRSGARQGQASAQGRAGSQGQAQGRVGSSADRQGRRGVSESQASDSEGHSDFSEGQAVGAHRQSGAGQRHEQRSSRGQHGSGFYPVYYYYEQEHSEEESDSQHQHGHQHEQQRGHQHQHQHQHEHEQPESGHRQQQFSGRGHQGAHQEQGRDSARSRGSNQGHSSSRHQADSPRVSARSGSGGRGQSPDASGRSSNRRDRPRQPSPSQSSDSQVILESRSKAGAGSPHLPTGGPDPAPAQGSRGPLQVDWQLTPPGALGRVKARHLPRVAQGHKAKHRAASARQLTGKGVEGSARVRPATARATLTSQKARQQQQSSGRGNQGAHQEQGRDSARSRGSNQGHSSSRHQADSPRVSARSGSGGRGQSPDASGRSSNRRDRPRQPSPSQSSDSHVHSGVQVEGRRGQSSSANRRAGSSSGSGVQGASAGGLAADASRRSGARQGQASAQGRAGSQGQAQGRVGSSADRQGRRGVSESQASDSEGHSDFSEGQAVGAHRQSGAGQRHEQRSSRGQHGSRYYYEQEHSEEESDSQHQHGHQHEQQRGHQHQHEHEQPESGHRQQQSSGRGHQGAHQEQGRDSARSRGSNQGHSSSRHQADSPRVSARSGSGGRGQSPDASGRSSNRRDRPRQPSPSQSSDSQVHSGVQVEGRRGQSSSANRRAGSSSGSGVQGASAGGLAADASRRSGARQGQASAQGRAGSQGQAQGRIGSSADRQGRRGVSESQASDSEGHSDFSEGQAVGAHRQSEAGQRHEQRSSRGQHGSGYYYEQEHSEEESDSQHQHGHQHEQQRGTQHQHEHQQPESGHRQQQSSGRGHQGTHQEQGRDSARSRGSNQGHSSSRHQADSPRVSARSGSGGRGQSPDASGRSSNRRDRPRQPSPSQSSDSQVHSGVQVEGRRRQSSSANRRAGSSSGSGVQGASAGGLAADASRRSGARQGQASAQGRAGSQGQAQGRVGSSADRQGRRGVSESQASDSEGHSDFSEGQAVGAHRQSGAGQRHEQRSSRGQHGSGFYPVYYYYEQEHSEEESDSQHQHGHQHEQQRGHQHQHQHEHEQPESGHRQQQSSGRGHQGAHQEQGRDSARSRGSNQGHSSSRHQADSPRVSARSGSGGRGQSPDASGRSSNRRDRPRQPSPSQSSDSQVHSGVQVEGRRGQSSSANRRAGSSSGSGVQGASAGGLAADASRRSGALQGQASAQGRAGSQGQAQGRVGSSADRQGRRGVSESQASDSEGHSDFSEGQAVGAHRQSGAGQRHEQRSSRGQHGSGYYYEQEHSEEESDSQHQHGHQHEQQRGHQHQHQHQHEHEQPESGHRQQQSSGRGNQGAHQEQGRDSARSRGSNQGHSSSRHQADSPRVSARSGSGGRGQSPDASGRSSNRRDRPRQPSPSQSSDSHVHSGVQVEGRRGQSSSANRRAGSSSSSGVQGASAGGLAADASRRSGARQGQASAQGRAGSQGQAQGRVGSSADRQGRRGVSESQASDSEGHSDFSEGQAVGAHRQSGAGQRHEQRSSRGQHGSGFYPVYYYYEQEHSEEESDSQHQHGHQHEQQRGHQHQHQHQHEHEQPESGHRQQQFSGRGHQGAHQEQGRDSARSRGSNQGHSSSRHQADSPRVSARSGSGGRGQSPDASVRSSNRRDRPRQPSPSQSSDSHVHSGVQVEGRRGQSSSANRRAGSSSGSGVQGASAGGLAADASRRSGARQGQASAQGRAGSQGQAQGRVGSSADRQGRRGVSESQASDSEGHSDFSEGQAVGAHRQSGAGQRHEQRSSRGQHGSGFYPVYYYYEQEHSEEESDSQHQHGHQHEQQRGHQHQHKHEHEQPESGHRQQQFSGRGHQGAHQEQGRDSARSRGSNQGHSSSRHQADSPRVSARSGSGGRGQSPDASGRSSNRRDRPRQPSPSQSSDSQVHSGVQVEGRRGQSSSANRRAGSSSSSGVQGASAGGLAADASRRSGARQGQASAQGRAGSQGQAQGRVGSSADRQGRRGVSESQASDSEGHSDFSEGQAVGAHRQSGAGQRHEQRSSRGQHGSGFYPVYYYYEQEHSEEESDSQHQHGHQHEQQRGHQHQHQHQHEHEQPESGHRQQQFSGRGHQGAHQEQGRDSARSRGSNQGHSSSRHQADSPRVSARSGSGGRGQSPDASGRSSNRRDRPRQPSPSQSSDSQVHSGVQVEGRRGQSSSANRRAGSSSGSGVQGASAGGLAADASRRSGARQGQASAQGRAGSQGQAQGRVGSSADRQGRRGVSESQASDSEGHSDFSEGQAVGAHRQSGAGQRHEQRSSRGQHGSGYYYEQEHSEEEQQQFSGRGHQGAHQEQGRDSARSRGSNQGHSSSRHQADSPRVSARSGSGGRGQSPDASGRSSNRRDRPRQPSPSQSSDSQVHSGVQVEGRRGQSSSANRRAGSSSGSGVQGASAGGLAADASRRSGARQGQASAQGRAGSQGQAQGRVGSSADRQGRRGVSESQASDSEGHSDFSEGQAVGAHRQSGAGQRHEQRSSRGQHGSGFYPVYYYYEQEHSEEESDSQHQHGHQHEQQRGHQHQHQHEHEQPESGHRQQQSSGRGHQGAHQEQGRDSARSRGSNQGHSSSRHQADSPRVSARSGSGGRGQSPDASGRSSNRRDRPRQPSPSQSSDSQVHSGVQVEGRRGQSSSANRRAGSSSGSGVQGTSAGGLAADASRRSGARQGQASAQGRAGSQGQAQGRVGSSADRQGRRGVSESQASDSEGHSDFSEGQAVGAHRQSGAGQRHEQRSSRGQHGSGYYYEQEHSEEESDSQHQHGHQHEQQRGHQHQHQHQHEHEQPESGHRQQQSSGRGNQGAHQKQGRDSARSRGSNQGHSSSRHQADSPRVSARSGSGGRGQSPDASGRSSNRRDRPRQPSPSQSSDSHVHSGVQVEGRRGQSSSANRRAGSSSGSGVQGASAGGLAADASRRSGARQGQASAQGRAGSQGQAQGRVGSSADRQGRRGVSESQASDSEGHSDFSEGQAVGAHRQSGAGQRHEQRSSRGQHGSGFYPVYYYYEQEHSEEESDSQHQHGHQHEQQRGHQHQHQHQHEHEQPESGHRQQQSSGRGHQGAHQEQGRDSARSRGSNQGHSSSRHQADSPRVSARSGSGGRGQSPDASGRSSNRRDRPRQPSPSQSSDSQVHSGVQVEGRRGQSSSANRRAGSSSGSGVQGASAGGLAADASRRSGARQGQASAQGRAGSQGQAQGRVGSSADRQGRRGVSGSQASDSEGHSDFSEGQAVGAHRQSGAGQRHEQRSSRGQHGSGYYYEQEHSEEESDSQHQHGHQHEQQRGHQHQHQHQHEHEQPESGHRQQQFSGRGHQGAHQEQGRDSARSRGSNQGHSSSRHQADSPRVSARSGSGGRGQSPDASGRSSNRRDRPRQPSPSQSSDSQVHSGVQVEGRRGQSSSANRRAGSSSGSGVQGASAGGLAADASRRSGALQGQASAQGRAGSQGQAQGRVGSSADRQGRRGVSESQASDSEGHSDFSEGQAVGAHRQSGAGQRHEQRSSRGQHGSGYYYEQEHSEEESDSQHQHGHQHEQQRGHQHQHQHQHEHEQPESGHRQQQSSGRGHQGAHQEQGRDSARSRGSNQGHSSSRHQADSPRVSARSGSGGRGQSPDASGRSSNRRDRPRQPSPSQSSDSQVHSGVQVEGRRGQSSSANRRAGSSSSSGVQGASAGGLAADASRRSGARQGQASAQGRAGSQGQAQGRVGSSADRQGRRGVSESQASDSEGHSDFSEGQAVGAHRQSGAGQRHEQRSSRGQHGSGFYPVYYYYEQEHSEEESDSQHQHGHQHEQQRGHQHQHQHQHEHEQPESGHRQQQFSGRGHQGAHQEQGRDSARSRGSNQGHSSSRHQADSPRVSARSGSGGRGQSPDASGRSSNRRDRPRQPSPSQSSDSQVHSGVQVEGRRGQSSSANRRAGSSSGSGVQGASAGGLAADASRRSGARQGQASAQGRAGSQGQAQGRVGSSADRQGRRGVSESQASDSEGHSDFSEGQAVGAHRQSGAGQRHEQRSSRGQHGSGYYYEQEHSEEESDSQHQQGHQHEQQRGHQHQHQHQHEHEQPESGHRQQQSSGRGHQGAHQEQGRDSARSRGSNQGHSSSRHQADSPRVSARSGSGGRGQSPDGSGRSSNRRDRPRQPSASQSSDSQVHSGVQVEAQRGQSSSANRRAGSSSGSGVQSAAASGQGGYESIFTAKHLDFNQSHSYYYY

SEQ ID NO: 11 - protein, 336 aa, Mus musculus; identical to SEQ ID NO: 7

SEQ ID NO: 12 - protein, 357 aa, Mus musculus
MSALLESITSMIEIFQQYSTSDKEEETLSKEELKELLEGQLQAVLKNPDDQDIAEVFMQMLDVDHDDKLDFAEYLLLVLKLAKAYYEASKNESFQTHGSNGRSKTDYKGLEEEGEEGNKQNLRRRHGGTDGKRKSDRTRSPNGKRGKRQESRCRSEGKDKHRREPEKHRHQQDSKRKQRHGSGSTERKDNRNKKNRQSKERNYDEIYDNGKYNEDWEASYNNCYYKTQNTTLDQREGNRRPRADSQKEPQSSHGQADNSDSEGGRQQSHSKPSPVRADQRRSRAGQAGSSKVSARSGSGGRGQSPDGSGRSSNRRDRPRQPSPSQSSDSQVHSGVQVEGRRGQSSSANRRAGSSSGS

SEQ ID NO: 13 - protein, 687 aa, Rattus norvegicus
MNRNENMNTNSQSPATGSRGPVGERTGQLAMNRKATAPGKGALTRRTAPLAPRRRSHAEGLEPVPVRVRGPRGRLPGTALSTPSPEGARPSAVDAQDTPLGEPTKTATSRQQTALPAPGPGEARPAPTVRARPPVVRPAAEALQPPGTHLAPNSLQTLLAGPDPAVDSSPPNDMLTQPRAAQEPAPEEEESPQLASSPPTEPGTSNPGGVEPGRPAPASPVTAKAILEPMPGSGKGRPQPLTGGQAPAQGASGPLLVAKQLTPPVAQGPVKARHQARVVQGPEAGKLRASLVMGSRQTATGTLGPGKHKPTQPQALTAGGLAGPARVRPATARATPTTQKHTHRGAHGGIQTSQRHEQRPSRGQQGSGHPQVYYYGVEETEDESDAQQGHHQQQQQQRQQQRQRHQHEQEREHEHQQPESSHRQQGSSGRTHRAARHEQESDSTRQRGSHQAHSSARTQEEIARGRSGASASEGPGPQREAARDSSEHAQSRRSETISRGRSGHSTGRAHEDRHEQATDRSARSGSRGGQAGSHSESEASGGQAGRRGTAATRHTSRPEQSPDTAGRTGSSRGQQSAQRHADSTPGSTRTGSRGRGESPAGQQSPDRARHIESRRGRTREASASQSSDSEGHSGAHAGIGQGQTSTTHRRAGSSSGSQQASVEGSDGYDSIVKSKYLSFSQSHCYYY

SEQ ID NO: 14 - protein, 3088 aa, Pan troglodytes
MSTLLENIFAIINLFKQYSKKDKNTDTLSKKELKELLEKEFRQILKNPDDPDMVDVFMDHLDIDHNKKIDFTEFLLMVFKLAQAYYESTRKENLPISGHKHRKHSHHDKHEDNKQEENKENRKRPSSLERRNNRKGNKGRSKSPRETGGKRHESSSEKKERKGYSPTHREEEYGKNHHNSSKKQKNKTENTRLEDNRKRLSERLEEKEDNEEGGYDYENTGRMTQKWIQSGHIATYYTIQDEAYDTTDNLLEENKIYERSRSSDDKSSSQVNRSRHENTSQVPLQESRTRKRRGSRVSQDRDSEGHSEDSERHSGSASRNHPGSARQQSRDGSRHPRSHDEDRASHGHSADSSRQSGTRHAETSSRGQTASSHEQARSSPGERHGSRHQQSADSSRHSATGRGQASSAVSDRGPRGSSGSQASDSEGHSENSDTQSVSGHGKAGPRQQSHQESARGRSGERSGHSGSFLYQVSTHEQSDSAHGRTGTSTGGRQGSHHEQARDSSRHSASQEGQDTIRGHPGSSRGGRQGSHHEQLVNRSGHSGSHHSHTTSQGRSDASHGQSGSRSASRQTRNEEQSGDGSRHSGSRHHEASSQADSSRHSQVGQGQSSGPRTSSHQGSSVSQDSDSEGHSEDSERWSGSASRNHHGSAREQSRDGSRHPRSHHEDRAGHGHSADSSRQSGTRHTESSSRGQAVSSHEQARSSPGERHGSRHQQSADSSRHSGIGHGQASSAVRDSGHRGSSGSQAIDSEGHSEDSDTQSVSSHGQAGPHQQSHKESARGQSGESSGRSGSFLYQVSSHEQSESTYGQTAPSTGGRQGSRHEQARNSSRHSASQDGQDTIRGHPGSSRGGRQGSYHEQSVDRSGHSGYHHSHTTPQGRSDASHGQSGPRSASRQTRNEEQSGDGSRHSGSRHHEPSTRASSSRHSQVGQGESAVSKTSRRQGSSVSQDRDSEGHSEDSERQSESASRNHYGSAREQSRHGSRNPRSHQEDRASHGHSAESSRQSGTHHAETSSHGQAASSQEQARSSRGERHGSRHQQSADSSTDSGTGGRQASSVVGDSGNRGSSGSQASDSEGHSEDSDTQSVSAHGQAGPRQQSHQESTRGQSGERSGRSGSFLYQVSTHEQSESAHGRTGPSTGGRQRSRHEQARDSSRHSASQESQDIIHAHPGSSRGGRQGSHYEQSVDRSGHSGSHHSHTTSQERSNASHGQSGSRSASRQTRNEEQSGDGSRHSGSRHHEASSRADSSRHSQVGQGQSSGPRTSRNQGSSVSQDSDSQGHSEDSERWSGSASRNHHGSAWEQSRDGSRHPGSHQEDRAGHGHSADSSRQSGTHHTESSSRGQAASSHEHARSSAGERHGSHHQQSADSSRHSGIGHGQASSAVRDSGHRGSSGSQASDSEGHSEDSDTQSLSAHGQAGPHQQSHQESTRGRSAERSGRSGSFLYQVSTHEQSESAHGRTGTSTGGRKRSLHEQARDSSRHSVSQEGQDTIHGHAGSSSGGRQGSHYEQLVDRSGHSGSHHSHTTSQGRSDAYHGQSGSRSASRQTHNDEQSGDGFRHSGSHHHEASSRADSSRHSQVGQGQSEGPRTSRHRESSVSQDSDSEGHSEDSERWSGSASRNHHGSAREQSRDGSRHPRSHHEDRAGHGHSADSSRQSGTRHTQTSSGGQAASSHEQGRSSAGERHGSRHQQSADSSRHSGIGHGQASSAVRDSGHRGYSGSQASDSEGHSEDSDTQSVSAHGQAGSHQQSHQESARGRSGERSGRSGSFLYQVSTHEQSESSHGWTGPSTRGRQGSRHEQAQDSSRHSASQEGQDTIRGHPGPSRGGRQGYHHEQSVDSSGHSGSHHSHITSQGSSHASHGQSGSRSASRTTRNDEQSVDGSRHSGSRHHEASTHADISRHSQAGQGQSEGSRTSRRQGSSVSQDSDSEGHSEDSERWSGSASRNHRGSAQEQSRDGSRHPRSHHEDRAGHGHSADSSRQSGTHHAETSSGGQAASSREQARSSPGERHGSRHQQSADSSRHSGIRRGQASSAVRDSGHWGSSGSQASDSEGHSEESDTQSVSGHGQDGPHQQSHQESARDRSGGRSGRSGSFLYQVSTHEQSESTHGQTGTSTGGRQGSHHEQARDSSRHSASQEGQDTIHAHPGSSRGGRQGSHHEQSVDTSGHSGSHHSHTTSQGRSDASHGQSGSRSASRQTRNDEQSGDGSRHSGSHHHEAFTQADSSRHSQSGQGESAGSRRSRRQGSSVSQDSDSQGHSEDSERWSGSASRNQHGSAREQSRDGSRHPGSHQEDRAGHGHSADSSRQSGTRHTESSSRGQAASSHEQARSSAGERHGSRHQLQSADSSRHSGIGHGQASSAVRDSGHRGSSGSQAIDSEGHSEDSDTQSVSAQGQAGPHQRSHKESARGQSGESSGRSGSFLYQVSTHEQPESTHGQSAPSTGGRQGSHHDQAQDSSRHSASQEGQDTIRGHPGPSRGGRQGSHHKQSVDRSGHSGSHHSHTTSQGRSDASRGQSGSRSASRQTHDKEQSGDGSRHSGSRHHEASSWADSSRHSQAGQGQSEGSRTSRRQGSSFSQDSDSEGHSEDSERRSGSASRNHRGSAQEQSRDGSRHPRSHHEDRAGHGHSADSSRQSGTHHAQNSSGGQAASFHEQARSSAGERHGSHHQQSADSSRHSGIGHGQASSAVRDSGHRGSSGSQASDSEGHSEDSDTQSVSAHGQAGPHQQSHQESTRGRSAERSGRSGSFLYQVSTHEQSESAHGRTGPSTGGRQGSRHEQARDSSRHSASQEGQDTIHGHPGSRRGGRQGSYHEQSVDRSGHSGSHHSHTTSQGRSDASHGQSGSRSASRQTRNEQQSGDGSRHSGSSHHEASTQADSSRHSQSGQGESAGSRRSRRQGSSVSQDSDSEAYPEDSERRSESASRNRHGSSREQSRDGSRHPGSSHRDTTRHVQSSPVQSDSSTAKEHGHFSSLSQDSAYRSGIQSRGSPHSSSSYHYQSEGTERQKGQSGLVWRHGSYGSADYDYGESGFRHSQHGSVSYNSNPVVFKERSDICKASAFGKDHPRYYATYINKDPGLCGHSSDISKQLGFSQSQRYYYYE

SEQ ID NO: 15 - protein, 2764 aa, Pan troglodytes
MSTLLENIFAIINLFKQYSKKDKNTDTLSKKELKELLEKEFRQILKNPDDPDMVDVFMDHLDIDHNKKIDFTEFLLMVFKLAQAYYESTRKENLPISGHKHRKHSHHDKHEDNKQEENKENRKRPSSLERRNNRKGNKGRSKSPRETGGKRHESSSEKKERKGYSPTHREEEYGKNHHNSSKKQKNKTENTRLEDNRKRLSERLEEKEDNEEGGYDYENTGRMTQKWIQSGHIATYYTIQDEAYDTTDNLLEENKIYERSRSSDDKSSSQVNRSRHENTSQVPLQESRTRKRRGSRVSQDRDSEGHSEDSERHSGSASRNHPGSARQQSRDGSRHPRSHDEDRASHGHSADSSRQSGTRHAETSSRGQTASSHEQARSSPGERHGSRHQQSADSSRHSATGRGQASSAVSDRGPRGSSGSQASDSEGHSENSDTQSVSGHGKAGPRQQSHQESARGRSGERSGHSGSFLYQVSTHEQSDSAHGRTGTSTGGRQGSHHEQARDSSRHSASQEGQDTIRGHPGSSRGGRQGSHHEQLVNRSGHSGSHHSHTTSQGRSDASHGQSGSRSASRQTRNEEQSGDGSRHSGSRHHEASSQADSSRHSQVGQGQSSGPRTSSHQGSSVSQDSDSEGHSEDSERWSGSASRNHHGSAREQSRDGSRHPRSHHEDRAGHGHSADSSRQSGTRHTESSSRGQAVSSHEQARSSPGERHGSRHQQSADSSRHSGIGHGQASSAVRDSGHRGSSGSQAIDSEGHSEDSDTQSVSSHGQAGPHQQSHKESARGQSGESSGRSGSFLYQVSSHEQSESTYGQTAPSTGGRQGSRHEQARNSSRHSASQDGQDTIRGHPGSSRGGRQGSYHEQSVDRSGHSGYHHSHTTPQGRSNASHGQSGSRSASRQTRNEEQSGDGSRHSGSRHHEASSRADSSRHSQVGQGQSSGPRTSRNQGSSVSQDSDSQGHSEDSERWSGSASRNHHGSAWEQSRDGSRHPGSHQEDRAGHGHSADSSRQSGTHHTESSSRGQAASSHEHARSSAGERHGSHHQQSADSSRHSGIGHGQASSAVRDSGHRGSSGSQASDSEGHSEDSDTQSLSAHGQAGPHQQSHQESTRGRSAERSGRSGSFLYQVSTHEQSESAHGRTGTSTGGRKRSLHEQARDSSRHSVSQEGQDTIHGHAGSSSGGRQGSHYEQLVDRSGHSGSHHSHTTSQGRSDAYHGQSGSRSASRQTHNDEQSGDGFRHSGSHHHEASSRADSSRHSQVGQGQSEGPRTSRHRESSVSQDSDSEGHSEDSERWSGSASRNHHGSAREQSRDGSRHPRSHHEDRAGHGHSADSSRQSGTRHTQTSSGGQAASSHEQGRSSAGERHGSRHQQSADSSRHSGIGHGQASSAVRDSGHRGYSGSQASDSEGHSEDSDTQSVSAHGQAGSHQQSHQESARGRSGERSGRSGSFLYQVSTHEQSESSHGWTGPSTRGRQGSRHEQAQDSSRHSASQEGQDTIRGHPGPSRGGRQGYHHEQSVDSSGHSGSHHSHITSQGSSHASHGQSGSRSASRTTRNDEQSVDGSRHSGSRHHEASTHADISRHSQAGQGQSEGSRTSRRQGSSVSQDSDSEGHSEDSERWSGSASRNHRGSAQEQSRDGSRHPRSHHEDRAGHGHSADSSRQSGTHHAETSSGGQAASSREQARSSPGERHGSRHQQSADSSRHSGIRRGQASSAVRDSGHWGSSGSQASDSEGHSEESDTQSVSGHGQDGPHQQSHQESARDRSGGRSGRSGSFLYQVSTHEQSESTHGQTGTSTGGRQGSHHEQARDSSRHSASQEGQDTIHAHPGSSRGGRQGSHHEQSVDTSGHSGSHHSHTTSQGRSDASHGQSGSRSASRQTRNDEQSGDGSRHSGSHHHEAFTQADSSRHSQSGQGESAGSRRSRRQGSSVSQDSDSQGHSEDSERWSGSASRNQHGSAREQSRDGSRHPGSHQEDRAGHGHSADSSRQSGTRHTESSSRGQAASSHEQARSSAGERHGSRHQLQSADSSRHSGIGHGQASSAVRDSGHRGSSGSQAIDSEGHSEDSDTQSVSAQGQAGPHQRSHKESARGQSGESSGRSGSFLYQVSTHEQPESTHGQSAPSTGGRQGSHHDQAQDSSRHSASQEGQDTIRGHPGPSRGGRQGSHHKQSVDRSGHSGSHHSHTTSQGRSDASRGQSGSRSASRQTHDKEQSGDGSRHSGSRHHEASSWADSSRHSQAGQGQSEGSRTSRRQGSSFSQDSDSEGHSEDSERRSGSASRNHRGSAQEQSRDGSRHPRSHHEDRAGHGHSADSSRQSGTHHAQNSSGGQAASFHEQARSSAGERHGSHHQQSADSSRHSGIGHGQASSAVRDSGHRGSSGSQASDSEGHSEDSDTQSVSAHGQAGPHQQSHQESTRGRSAERSGRSGSFLYQVSTHEQSESAHGRTGPSTGGRQGSRHEQARDSSRHSASQEGQDTIHGHPGSRRGGRQGSYHEQSVDRSGHSGSHHSHTTSQGRSDASHGQSGSRSASRQTRNEQQSGDGSRHSGSSHHEASTQADSSRHSQSGQGESAGSRRSRRQGSSVSQDSDSEAYPEDSERRSESASRNRHGSSREQSRDGSRHPGSSHRDTTRHVQSSPVQSDSSTAKEHGHFSSLSQDSAYRSGIQSRGSPHSSSSYHYQSEGTERQKGQSGLVWRHGSYGSADYDYGESGFRHSQHGSVSYNSNPVVFKERSDICKASAFGKDHPRYYATYINKDPGLCGHSSDISKQLGFSQSQRYYYYE

SEQ ID NO: 16 - protein, 1183 aa, Macaca mulatta
MSTLLENIFAIINLFKQYSKKDKNTDTLSKKELKELLEKEFRPILKNPDDPDTVEVFMDHLDIDHNKKIDFTEFLLMVFKLAQAYYESTRKQNLPIAGHKHRKHSHHDKHEDNKEEENKEKRKRPLSLERRNNRKGNTGRSKSPRERGGKRHESSFEKKERKGYSPTYEEEEYGQNHHKSSKKEKNKTEITRLEHEGKRISERPEKKEEKEDGQFDYENAGRMDEKWTESGHIAIYHAIQDEVDDTTENILEENRRYETSRSPHDKSSLRVNRSPNANTSQIPLVEPRRRTRQRSSVSQDSDSEGHSEDSERQSESASRNHHGSVREQSRHGSRHPGSHHEDRAGHGHSADSSTQSGTRHTETSSRGQAVSSHEQARSSPGERHGSRHQQSAESSRHSGIGRGQASSAVSDRGHQGPSGSHFSDSEGHSEHSDTQSVSGHGQAGPHPHSHQESARGRSRERSGRSGSFLYQVSTHEQSESTHGRTGPSSAGRQGSRNEQARDSSRHSASHEVQDTVHGHHGSSRGRRQGSHHEQLVDSSGHSGSHHSHTTSQGRSDASRGESGARSASRQTRHEEQSGDGSRHSGSRHHESSNRADSSRHAQSSQGQSAGFRTSTRRGSSVSQDSDSEGHSEDSERQSESASRNHHGSVREQSRHGSGHSGSHHQDKVGHRYSGDSSRQSGTHHVETSSHGQAASSHEQTRSSPGERHGSHHQQSADSSRHSGTGRGQASSAVSDRGHQGPSGSHFSDSEGHSEHSDTQSVSGQGQAGRHPHSHQESARGRSGERSGRSGSFVYQVSTHEQSESTHGRTGPSTGGRQGSRNEQARDSSRHSVSHEGQDTIHGHHGSSRGGRQGSHHEQSVDSSGHSGSHHSHTTSQGRSDASRGESGARSASRQTRHEEQSGDGSRHSGSRHHEASNRADSSRHAQSGQGQSAGFRTSTRRGSSVSQDSDSEGHSEDSERQSESASRNHHGSVREQSRHGSRHPGSHHEDRAGHGHSADSSRQSGTRHTETSSRGQAVSSHEQARSSPGERHGSRHQQSAESSRHSGIGRGQASSAVSDRGHQGPSGSHFSDSEGHSEHSDTQSVSGHGQAGPHPHSHQESARGRSGERSGRSGSFLYQVSTHEQSESTHGRTGPSSAGRQGSRNEQARDSSRHSASHEVQDTVHGHHGSSRGGRQGSHHEQS

SEQ ID NO: 17 - protein, 2949 aa, Macaca mulatta
  REGION 2160..2164: note = misc_feature - Xaa can be any naturally occurring amino acid
MTDLLRSVVTVIDVFYKYTKQDGECGTLSKDELKELLEKEFHPVLKNPDDPDTVDVIMHMLDRDHDRRLDFTEFLLMIFKLTMACNKVLSKEYCKASGSKKHRRGHRHQEEESETEEDEEDTPEHKSGYRHSSWSEGEEHGYSSGHSRGTVKRRHGSNSRRLGRQGHLSSSGNQERSQKRYHRSSSGHSWSSGKERHGFSSGELRERINKSHVSPSREFGEEYESGSGSKSWERKGHGGLSCGLEISGHESNSTQSRSSGQKLGSSRSCSGDSRRRSHACGYSNSSGCGRPQNASNSCQHRFGGQVNQSSYIQSGCQSGINGEQGHDCVSGGQPSGCGQPESNSCSQSYSQRGYGARENGQPQNCGGQQRTGSSQSSFCGQYESGGSQSCSNGQHEHGSCGRFSNSSSSNEFSKCGKHRSGSGQFTSCEQHGTGLSQSSGFEQQVAGSSQTCSQYGSRSSQSSGYDEHGSSSGKTSGFGQHRSGSGHSSGFGQHGSGSGQSFGFGQHGSGSGQSSGFGQHESRSCQSSYGQHGSGSSQSSGYGQHASRQTSGFGQHGLGSGQSTGFGQYGSGSGQSSGFGQHGSGSGQSSGFGQHESRSGQSSYGQHSSSSSQSSGYGQHGSRQTSGFGQHGSGSGQSTGFGQYGSSLGQSSGFGQHGSGSGQSSGFGQHESTSGQSSYGQHGFGSSQSSGCGQHGLSSGQTSGFGQHELSSGQSSSFGQHGSGSGQSSGFRQHESGSGQSSGFGQHESRSHQSSYGPHGSGSGQSSGYGQHGSSSGQTSGFGQQGSSSSQYSGFGQHGSGLGQSSGFGQHGTGSGQFSGFGQHESRSHQSSYGQHGSGSSQSSGYGQHGSSSGHTTGFGQHRSSSGQYSGFGQHGSGLGQSSGFGQHGTGSGQSSFGQHESRSHQSSYGQHGSGSSQSSSYGQHGSSSGQTSGFGQHRSGSGQSSGFGQYGLGSGSGFGQHGSGTGQSSGFARHEYRSGQSSYGQHGTGSSQSSGCGQRESGSGPTTGFGQHVSGSDNFSSSGQHISGSDQSTGFGQYGSGSGQSTGLGQVESQQVASGSTVHGRQETTHGQTINTARHSQSGQGQSTQTGSRVSRRRRSSQSENIDSEVHSRVSHRHSEHIDTQVGSHYPESGSTVHRRQGTTHGQRGDTTRHSHSGHGQSTQTGSRTTGRQRFSHSDATDSEVHSGVSHRPHSQEHTHGQDGSQLGESQSTVHERHETTYGQTGDATGHGYSGHGQSTQIGSRTSGRRGSGHSESSDTEVHSGGSHRPHSQEQTHGQARSQHGESRSTVHERHGTTHGQTGDTTRYAHYHNGQSAQRGSRTTGRGSGHSEYSDSELYSGGSHTYSGHTHGQAGSQHGESDSIVHERYGTTHGQTGDTTRHAHYSHGQSKQRGSRTTGRRGSGHSEYSDSEGHSGGSHTHSGHTHGHTHGQAGSQHGESGSSGHGGQGTTHGQTGDTTRHAHYGHGQSTQRGSRTAGRRGSGHSEYSDSEGHSGVSHTHSGHTHGQAGSQHGESESTVHERQQTTHGQTGDTTRHAHYGHGQSTQTGSRTTGRRGSGHSEYSDSEGHSGVSHTHSGHTHGQARSQHGESGSAIHGRQGTIHGQTGDTTRHGQSGHGQSTQTGSRTTGRRGSGHSEYSDSEGHSGGSHTHSGHTHGQAGSQHGESGSTVHGRQGTIHGQTGDTTRHGQSGHGQSIETGSRTTGRRGSGHSEYSDSEGHSGVSHTHSGHTHGQAGSQHGESESTVHERQQTTHGQTGDITEHGHSSHGQTTQTGSRTTGRRGSGHSEYSDSEWHSGSHTHSGHTHGQAGFQHGESGSAVHGRQGTIHGQTGDTTRHGQSGHGESIQTGSRTIGRRGSGHSEYSDSEGHSGISHTHSGHTHGQAGSQHGESGSSGHGRQGTAHGQTGDTTRHAHYDHGQSTQRGSRTAGRRGSGHSEYSDSEGHSGVSHTHSGHTHGQAGSQHGESGAAVHGRQGIIHGQTGDTTRHGQSGQGQSTQRGSRTTGRRGSGHSEYSDSVGHSGVSHTHSGHTHGLAGSQHGESGSSGHGRQGTLHGQTGDTTRHAHYGHGQSTQRGSRTAGRRGSGHSEYSDSEWHSGGSHTHSGHTHGQAGSQHGESGSAVHGRQGTIHGQTGDTTRHGQSGHGQSTQIGSRTTGRRGSGHXXXXXRHTETSSRGQAVSSHEQARSSPGERHGSRHQQSAESSRHSGIGRGQASSAVSERGHQGPSGSLFSDSEGHSEHSDTQSVSGHGQAGPHPHSHQESARGRSGERSGRSGSFLYQVSTHEQSESTHGWTGPSSAGRQGSRNEQARDSSRHSVSHEVQDTVHGHSGSSRGRRQGSHHEQLVDSSGHSGSHHSHTTSQGRSDASRGESGARSASRQTRHEEQSGDGSRHSGSRHHEASNRADSSRHAQSGQGQSAGFRTSTRRGSSVSQDSDSEGHSEDSERQSESASRNHHGSVREQSRHGSRYPGSHHEDGAGHGHTADSPRQSGTHHVETSSHGQAASSHEQTRSSPGERHGSRHQQSAESSRHSGIGRGQASSAVSERGHQGPSGSQFSDSEGHSEHSDTQSVSGHGQAGPHPHSHQESARGRSGERSGRSGSFVYQVSTHEQSESTHGQTGPSTGGRQGSRNEQARDSSRHSVSHEGQDTIHGHSESSIGGRQGSHHEQSVDSSGHSGSHHSHTTSQGRSDASRGQSGSRSASRQTRHEEQSGDGYRHSGSRLHEASTQADSFRHSHSGQGQSAGSRRSTLRGSSVNQDSASEGHSEDSERQSESASRNPHGAVREQSRDVSRHPRSYHHDTGNHVQSSSVYSDTTTSKEHGHFGSLSQDSAYHSGIQSRGSPHSSSSYNYHSEGTERERGQSGLVWRHGSYGSADYDYGESRFRHSQHGSVSYNSNPVVFKERSDIRKASAFGEDHPRYYARYVNRQPGLYRHSSDISKQLGFSQSQRYYYYE

SEQ ID NO: 18 - protein, 25 aa, Staphylococcus epidermidis
MKKLAFAITAASGAAAVLSHHDAEA

SEQ ID NO: 19 - protein, 30 aa, Staphylococcus epidermidis
WLDNRAFSKKFVPVVMATSVALFFLNLAFA

SEQ ID NO: 20 - protein, 29 aa, Staphylococcus epidermidis
MAKKFNYKLPSMVALTLFGTAFTAHQANA

SEQ ID NO: 21 - protein, 27 aa, Staphylococcus epidermidis
MKKRFLSICTMTIAALATTTMVNTSYA

SEQ ID NO: 22 - protein, 30 aa, Staphylococcus epidermidis
NLKKQSKLILIFICIFTFFIMIIQSQFLMG

SEQ ID NO: 23 - protein, 26 aa, Staphylococcus epidermidis
MKIFKLTSLTLAALTLAFPFSHVAQA

SEQ ID NO: 24 - protein, 28 aa, Staphylococcus epidermidis
MKKTVIASTLAVSLGIAGYGLSGHEAHA

SEQ ID NO: 25 - protein, 27 aa, Staphylococcus epidermidis
MKKNKFLVYLLSTALITPTFATQTAFA

SEQ ID NO: 26 - protein, 35 aa, Staphylococcus epidermidis
MKTRQNKYSIRKFSVGASSILIAALLFMGGGSAQA

SEQ ID NO: 27 - protein, 37 aa, Staphylococcus epidermidis
MKNNNETRRFSIRKYTVGVVSIITGITIFVSGQHAQA

SEQ ID NO: 28 - protein, 30 aa, Staphylococcus epidermidis
MKKKLSYMITIMLAFTLSLALGLFFNSAHA

SEQ ID NO: 29 - protein, 13 aa, Human immunodeficiency virus
GRKKRRQRRRPPQ

SEQ ID NO: 30 - protein, 27 aa, synthetic construct
GWTLNSAGYLLGKINLKALAALAKKIL

SEQ ID NO: 31 - protein, 18 aa, synthetic construct
KLALKLALKALKAALKLA

SEQ ID NO: 32 - protein, 30 aa, synthetic construct
WEAKLAKALAKALAKHLAKALAKALKACEA

SEQ ID NO: 33 - protein, 21 aa, synthetic construct
KETWWETWWTEWSQPKKKRKV

SEQ ID NO: 34 - protein, 9 aa, synthetic construct
RRRRRRRRR

SEQ ID NO: 35 - protein, 24 aa, synthetic construct
LGTYTQDFNKFHTFPQTAIGVGAP